European Patent Application EP 4 471 046 A1, published December 4, 2024. Title: 甾类化合物、其制备方法和应用. Applicant: 珂阑（上海）医药科技有限公司. The sequence listing filed with the application follows.

SEQUENCE LISTING (14 sequences)

SEQ ID NO: 1 - DNA, 20 bp, synthetic construct
  source 1..20: mol_type = other DNA
aactttggcattgtggaagg

SEQ ID NO: 2 - DNA, 20 bp, synthetic construct
  source 1..20: mol_type = other DNA
ggatgcagggatgatgttct

SEQ ID NO: 3 - DNA, 21 bp, synthetic construct
  source 1..21: mol_type = other DNA
gctgcggaaacttcaggaaat

SEQ ID NO: 4 - DNA, 23 bp, synthetic construct
  source 1..23: mol_type = other DNA
agagacgtgtcactcctggactt

SEQ ID NO: 5 - DNA, 20 bp, synthetic construct
  source 1..20: mol_type = other DNA
ccggagaccccttagatcga

SEQ ID NO: 6 - DNA, 26 bp, synthetic construct
  source 1..26: mol_type = other DNA
tagcctgtaaaagatttctgcaaacc

SEQ ID NO: 7 - DNA, 22 bp, synthetic construct
  source 1..22: mol_type = other DNA
cttgtggaatgccttgtgattg

SEQ ID NO: 8 - DNA, 19 bp, synthetic construct
  source 1..19: mol_type = other DNA
agccgaagcagcacatgat

SEQ ID NO: 9 - DNA, 18 bp, synthetic construct
  source 1..18: mol_type = other DNA
gccgtgaactgggtcgaa

SEQ ID NO: 10 - DNA, 25 bp, synthetic construct
  source 1..25: mol_type = other DNA
gcatatatagcaatgtctcctgcaa

SEQ ID NO: 11 - DNA, 21 bp, synthetic construct
  source 1..21: mol_type = other DNA
gtccctgaagtcagctgcata

SEQ ID NO: 12 - DNA, 21 bp, synthetic construct
  source 1..21: mol_type = other DNA
tgggacagtccagttcttcat

SEQ ID NO: 13 - DNA, 22 bp, synthetic construct
  source 1..22: mol_type = other DNA
tgctgacagaggcaccactgaa

SEQ ID NO: 14 - DNA, 23 bp, synthetic construct
  source 1..23: mol_type = other DNA
cagttgtacgtccagaggcatag